European Patent Application EP 4 296 358 A1, published December 27, 2023. Title: ANTI-TETRANOR-PGDM MONOCLONAL ANTIBODIES AND THEIR USES. Applicant: The University of Tokyo Tsuzuki Educational Institute. The sequence listing filed with the application follows.

SEQUENCE LISTING (84 sequences)

SEQ ID NO: 1 - protein, 8 aa, Mus musculus
  MISC_FEATURE (4)..(4): Xaa is F, A or S.
  MISC_FEATURE (6)..(6): Xaa is N or R.
  MISC_FEATURE (8)..(8): Xaa is A or W.
GYTXTXYX

SEQ ID NO: 2 - protein, 8 aa, Mus musculus
  MISC_FEATURE (2)..(2): Xaa is N or Y.
  MISC_FEATURE (4)..(4): Xaa is F or G.
  MISC_FEATURE (5)..(5): Xaa is N or D.
  MISC_FEATURE (6)..(6): Xaa is D or G.
  MISC_FEATURE (7)..(7): Xaa is G, N or D.
IXPXXXXT

SEQ ID NO: 3 - protein, 13 aa, Mus musculus
  MISC_FEATURE (2)..(2): Xaa is R, S or T.
  MISC_FEATURE (3)..(3): Xaa is Y or V.
  MISC_FEATURE (4)..(4): Xaa is Y or absent.
  MISC_FEATURE (5)..(5): Xaa is Y or absent.
  MISC_FEATURE (6)..(6): Xaa is Y or absent.
  MISC_FEATURE (7)..(7): Xaa is G or S.
  MISC_FEATURE (8)..(8): Xaa is S or R.
  MISC_FEATURE (9)..(9): Xaa is K or W.
  MISC_FEATURE (10)..(10): Xaa is A or F.
  MISC_FEATURE (11)..(11): Xaa is M or F.
  MISC_FEATURE (12)..(12): Xaa is D or A.
  MISC_FEATURE (13)..(13): Xaa is Y or V.
AXXXXXXXXXXXX

SEQ ID NO: 4 - protein, 9 aa, Mus musculus
  MISC_FEATURE (1)..(1): Xaa is T or S.
  MISC_FEATURE (5)..(5): Xaa is T or R.
  MISC_FEATURE (6)..(6): Xaa is T or I.
  MISC_FEATURE (8)..(8): Xaa is N, Y or K.
  MISC_FEATURE (9)..(9): Xaa is Y or H.
XGAVXXSXX

SEQ ID NO: 5 - protein, 9 aa, Mus musculus
  MISC_FEATURE (4)..(4): Xaa is Y, F or N.
  MISC_FEATURE (9)..(9): Xaa is V or I.
ALWXSNHWX

SEQ ID NO: 6 - DNA, 417 bp, Mus musculus
atggaatggagttggatatttctctttctcctgtcaggaactgcaggtgtccactctgaggtccagctgcagcagtctggacctgagctggtaaagcctggggcttcagtgaagatgtcctgcaaggcttctggatacacattcactaactatgctatgtactgggtgaagcagaaacctgggcagggccttgagtggattggatatattaatcctttcaatgacggtactaagaacaatgagaagttcaaaggcaaggccacactgacttcagacaaatcctccagcacagcctacatggagctcagcagcctgacctctgaggactctgcggtctattactgtgcaagatattattactacggtagcaaggctatggactactggggtcaaggaaccgcagtcaccgtctcctca

SEQ ID NO: 7 - protein, 139 aa, Mus musculus
MEWSWIFLFLLSGTAGVHSEVQLQQSGPELVKPGASVKMSCKASGYTFTNYAMYWVKQKPGQGLEWIGYINPFNDGTKNNEKFKGKATLTSDKSSSTAYMELSSLTSEDSAVYYCARYYYYGSKAMDYWGQGTAVTVSS

SEQ ID NO: 8 - DNA, 360 bp, Mus musculus
gaggtccagctgcagcagtctggacctgagctggtaaagcctggggcttcagtgaagatgtcctgcaaggcttctggatacacattcactaactatgctatgtactgggtgaagcagaaacctgggcagggccttgagtggattggatatattaatcctttcaatgacggtactaagaacaatgagaagttcaaaggcaaggccacactgacttcagacaaatcctccagcacagcctacatggagctcagcagcctgacctctgaggactctgcggtctattactgtgcaagatattattactacggtagcaaggctatggactactggggtcaaggaaccgcagtcaccgtctcctca

SEQ ID NO: 9 - protein, 120 aa, Mus musculus
EVQLQQSGPELVKPGASVKMSCKASGYTFTNYAMYWVKQKPGQGLEWIGYINPFNDGTKNNEKFKGKATLTSDKSSSTAYMELSSLTSEDSAVYYCARYYYYGSKAMDYWGQGTAVTVSS

SEQ ID NO: 10 - protein, 8 aa, Mus musculus
GYTFTNYA

SEQ ID NO: 11 - protein, 8 aa, Mus musculus
INPFNDGT

SEQ ID NO: 12 - protein, 13 aa, Mus musculus
ARYYYYGSKAMDY

SEQ ID NO: 13 - DNA, 384 bp, Mus musculus
atggcctggatttcacttatactctctctcctggctctcagctcaggggccatttcccaggctgttgtgactcaggaatctgcactcaccacatcacctggtgaaacagtcacactcacttgtcgctcaagtactggggctgttacaactagtaactatgccaactgggtccaagaaaaaccagatcatttattcactggtctaataggtggtaccaacaaccgagctccaggtgttcctgccagattctcaggctccctgattggagacaaggctgccctcaccatcacaggggcacagactgaggatgaggcaatatatttctgtgctctatggtacagcaaccattgggtgttcggtggaggaaccaaactgactgtccta

SEQ ID NO: 14 - protein, 128 aa, Mus musculus
MAWISLILSLLALSSGAISQAVVTQESALTTSPGETVTLTCRSSTGAVTTSNYANWVQEKPDHLFTGLIGGTNNRAPGVPARFSGSLIGDKAALTITGAQTEDEAIYFCALWYSNHWVFGGGTKLTVL

SEQ ID NO: 15 - DNA, 327 bp, Mus musculus
caggctgttgtgactcaggaatctgcactcaccacatcacctggtgaaacagtcacactcacttgtcgctcaagtactggggctgttacaactagtaactatgccaactgggtccaagaaaaaccagatcatttattcactggtctaataggtggtaccaacaaccgagctccaggtgttcctgccagattctcaggctccctgattggagacaaggctgccctcaccatcacaggggcacagactgaggatgaggcaatatatttctgtgctctatggtacagcaaccattgggtgttcggtggaggaaccaaactgactgtccta

SEQ ID NO: 16 - protein, 109 aa, Mus musculus
QAVVTQESALTTSPGETVTLTCRSSTGAVTTSNYANWVQEKPDHLFTGLIGGTNNRAPGVPARFSGSLIGDKAALTITGAQTEDEAIYFCALWYSNHWVFGGGTKLTVL

SEQ ID NO: 17 - protein, 9 aa, Mus musculus
TGAVTTSNY

SEQ ID NO: 18 - protein, 9 aa, Mus musculus
ALWYSNHWV

SEQ ID NO: 19 - DNA, 408 bp, Mus musculus
atggaatgtaactggatacttccttttattctgtcagtaacttcaggtgtctactcacgggttcagctccagcagtctggggctgaggtggctagacctggggcttcagtggaattgtcctgcaagtcttctggctacaccgcaactcgctactgggtgcagtggataagacagagacctgggcagggtctggaatggattggggccatttatcctggagatggtaatacttggtacactcagagattcaaggacaaggccgcattgactgtagataaaacctccagcactgcctacatgcgactcagcagcttgacatctgaggactctgcggtcttttactgtgcaagcgtctcccggtggttcttcgctgtctggggcgcagggaccacggtcaccgtctcctcg

SEQ ID NO: 20 - protein, 136 aa, Mus musculus
MECNWILPFILSVTSGVYSRVQLQQSGAEVARPGASVELSCKSSGYTATRYWVQWIRQRPGQGLEWIGAIYPGDGNTWYTQRFKDKAALTVDKTSSTAYMRLSSLTSEDSAVFYCASVSRWFFAVWGAGTTVTVSS

SEQ ID NO: 21 - DNA, 351 bp, Mus musculus
cgggttcagctccagcagtctggggctgaggtggctagacctggggcttcagtggaattgtcctgcaagtcttctggctacaccgcaactcgctactgggtgcagtggataagacagagacctgggcagggtctggaatggattggggccatttatcctggagatggtaatacttggtacactcagagattcaaggacaaggccgcattgactgtagataaaacctccagcactgcctacatgcgactcagcagcttgacatctgaggactctgcggtcttttactgtgcaagcgtctcccggtggttcttcgctgtctggggcgcagggaccacggtcaccgtctcctcg

SEQ ID NO: 22 - protein, 117 aa, Mus musculus
RVQLQQSGAEVARPGASVELSCKSSGYTATRYWVQWIRQRPGQGLEWIGAIYPGDGNTWYTQRFKDKAALTVDKTSSTAYMRLSSLTSEDSAVFYCASVSRWFFAVWGAGTTVTVSS

SEQ ID NO: 23 - protein, 8 aa, Mus musculus
GYTATRYW

SEQ ID NO: 24 - protein, 8 aa, Mus musculus
IYPGDGNT

SEQ ID NO: 25 - protein, 10 aa, Mus musculus
ASVSRWFFAV

SEQ ID NO: 26 - DNA, 384 bp, Mus musculus
atggcctggatttcacttatactctctctcctggctctcagctcaggggccatttcccaggctattgtgactcaggaatctgcactcaccacatcacctggtgaaacagtcacactcacttgtcgctcaagttctggggctgttacaactagtaaccacgccaactgggtccaagaaaaaccagatcatttattcactggtctaataggtgataccaacaaccgagctccaggtgttcctgccagattctcaggctccctgattggagacaaggctgccctcaccatcacaggggcacagactgaggatgaggcaatatatttctgtgctctgtggttcagcaaccactgggtgttcggtggaggaaccaaactgactgtccta

SEQ ID NO: 27 - protein, 128 aa, Mus musculus
MAWISLILSLLALSSGAISQAIVTQESALTTSPGETVTLTCRSSSGAVTTSNHANWVQEKPDHLFTGLIGDTNNRAPGVPARFSGSLIGDKAALTITGAQTEDEAIYFCALWFSNHWVFGGGTKLTVL

SEQ ID NO: 28 - DNA, 327 bp, Mus musculus
caggctattgtgactcaggaatctgcactcaccacatcacctggtgaaacagtcacactcacttgtcgctcaagttctggggctgttacaactagtaaccacgccaactgggtccaagaaaaaccagatcatttattcactggtctaataggtgataccaacaaccgagctccaggtgttcctgccagattctcaggctccctgattggagacaaggctgccctcaccatcacaggggcacagactgaggatgaggcaatatatttctgtgctctgtggttcagcaaccactgggtgttcggtggaggaaccaaactgactgtccta

SEQ ID NO: 29 - protein, 109 aa, Mus musculus
QAIVTQESALTTSPGETVTLTCRSSSGAVTTSNHANWVQEKPDHLFTGLIGDTNNRAPGVPARFSGSLIGDKAALTITGAQTEDEAIYFCALWFSNHWVFGGGTKLTVL

SEQ ID NO: 30 - protein, 9 aa, Mus musculus
SGAVTTSNH

SEQ ID NO: 31 - protein, 9 aa, Mus musculus
ALWFSNHWV

SEQ ID NO: 32 - DNA, 408 bp, Mus musculus
atggaatgtaactggatacttccttttattctgtcagtaacttcaggtgtctactcacaaattcagctccagcagtctggggctgaggtggcaagacctgggacttcaatgagattgtcctgcaaggcttctggctacacctttactcgctactggatgcagtgggtaaaacagaggcctggacagggtctggaatggattggggctatttatcctggagatggtaatacttggtatactcagaaattcaaggacaaggccacattgactatagataaaacctccggcacagcctacattcaactcatcagcttggcatctgaggactctgcggtctattactgtgcaacagtctcccggtggtttttcgctgtctggggcgcagggacaacggtcaccgtctcctca

SEQ ID NO: 33 - protein, 136 aa, Mus musculus
MECNWILPFILSVTSGVYSQIQLQQSGAEVARPGTSMRLSCKASGYTFTRYWMQWVKQRPGQGLEWIGAIYPGDGNTWYTQKFKDKATLTIDKTSGTAYIQLISLASEDSAVYYCATVSRWFFAVWGAGTTVTVSS

SEQ ID NO: 34 - DNA, 351 bp, Mus musculus
caaattcagctccagcagtctggggctgaggtggcaagacctgggacttcaatgagattgtcctgcaaggcttctggctacacctttactcgctactggatgcagtgggtaaaacagaggcctggacagggtctggaatggattggggctatttatcctggagatggtaatacttggtatactcagaaattcaaggacaaggccacattgactatagataaaacctccggcacagcctacattcaactcatcagcttggcatctgaggactctgcggtctattactgtgcaacagtctcccggtggtttttcgctgtctggggcgcagggacaacggtcaccgtctcctca

SEQ ID NO: 35 - protein, 117 aa, Mus musculus
QIQLQQSGAEVARPGTSMRLSCKASGYTFTRYWMQWVKQRPGQGLEWIGAIYPGDGNTWYTQKFKDKATLTIDKTSGTAYIQLISLASEDSAVYYCATVSRWFFAVWGAGTTVTVSS

SEQ ID NO: 36 - protein, 8 aa, Mus musculus
GYTFTRYW

SEQ ID NO: 37 - protein, 8 aa, Mus musculus
IYPGDGNT

SEQ ID NO: 38 - protein, 10 aa, Mus musculus
ATVSRWFFAV

SEQ ID NO: 39 - DNA, 384 bp, Mus musculus
atggcctggatttcacttatactctctctcctggctctcagctcaggggccttttcccaggctgttgtgactcaggaatctgcactcaccacatcacctggtgaaacagtcacactcacttgtcgctcaagtactggggctgttacaactagttatcatgccaactgggtccaagaaaaaccagatcatttattcactggtctaattggtgataccgacaaccgagctccaggtattcctgccaggttctcaggctccctgattggagacaaggctgccctcaccatcacaggggctcagcctgaggatgaggcaatctatttctgtgctctatggtacagcaaccactggatcttcggtggaggaaccaaactgactgtcctg

SEQ ID NO: 40 - protein, 128 aa, Mus musculus
MAWISLILSLLALSSGAFSQAVVTQESALTTSPGETVTLTCRSSTGAVTTSYHANWVQEKPDHLFTGLIGDTDNRAPGIPARFSGSLIGDKAALTITGAQPEDEAIYFCALWYSNHWIFGGGTKLTVL

SEQ ID NO: 41 - DNA, 327 bp, Mus musculus
caggctgttgtgactcaggaatctgcactcaccacatcacctggtgaaacagtcacactcacttgtcgctcaagtactggggctgttacaactagttatcatgccaactgggtccaagaaaaaccagatcatttattcactggtctaattggtgataccgacaaccgagctccaggtattcctgccaggttctcaggctccctgattggagacaaggctgccctcaccatcacaggggctcagcctgaggatgaggcaatctatttctgtgctctatggtacagcaaccactggatcttcggtggaggaaccaaactgactgtcctg

SEQ ID NO: 42 - protein, 109 aa, Mus musculus
QAVVTQESALTTSPGETVTLTCRSSTGAVTTSYHANWVQEKPDHLFTGLIGDTDNRAPGIPARFSGSLIGDKAALTITGAQPEDEAIYFCALWYSNHWIFGGGTKLTVL

SEQ ID NO: 43 - protein, 9 aa, Mus musculus
TGAVTTSYH

SEQ ID NO: 44 - protein, 9 aa, Mus musculus
ALWYSNHWI

SEQ ID NO: 45 - DNA, 408 bp, Mus musculus
atggaatgtaactggatacttccttttattctgtcagtaacttcaggtgtctactcacaggttcagctccagcagtctggggctgaggtggcaagacctggggcttcagtgaaattgtcctgcaaggcttctggctacacctttactcgctactggatgcagtggataaaacagaggcctggacagggtctggaatggattggggctatttatcctggagatggtgatacttggtatactcagaaattcaaggacaaggccacgttgactatagataaaacctccggcaccgcctacattcaactcatcagcttggcatctgaggactctgcggtctattactgtgcatcagtctcccggtggttcttcgctgtctggggcgcagggaccacggtcaccgtctcctca

SEQ ID NO: 46 - protein, 136 aa, Mus musculus
MECNWILPFILSVTSGVYSQVQLQQSGAEVARPGASVKLSCKASGYTFTRYWMQWIKQRPGQGLEWIGAIYPGDGDTWYTQKFKDKATLTIDKTSGTAYIQLISLASEDSAVYYCASVSRWFFAVWGAGTTVTVSS

SEQ ID NO: 47 - DNA, 351 bp, Mus musculus
caggttcagctccagcagtctggggctgaggtggcaagacctggggcttcagtgaaattgtcctgcaaggcttctggctacacctttactcgctactggatgcagtggataaaacagaggcctggacagggtctggaatggattggggctatttatcctggagatggtgatacttggtatactcagaaattcaaggacaaggccacgttgactatagataaaacctccggcaccgcctacattcaactcatcagcttggcatctgaggactctgcggtctattactgtgcatcagtctcccggtggttcttcgctgtctggggcgcagggaccacggtcaccgtctcctca

SEQ ID NO: 48 - protein, 117 aa, Mus musculus
QVQLQQSGAEVARPGASVKLSCKASGYTFTRYWMQWIKQRPGQGLEWIGAIYPGDGDTWYTQKFKDKATLTIDKTSGTAYIQLISLASEDSAVYYCASVSRWFFAVWGAGTTVTVSS

SEQ ID NO: 49 - protein, 8 aa, Mus musculus
GYTFTRYW

SEQ ID NO: 50 - protein, 8 aa, Mus musculus
IYPGDGDT

SEQ ID NO: 51 - protein, 10 aa, Mus musculus
ASVSRWFFAV

SEQ ID NO: 52 - DNA, 384 bp, Mus musculus
atggcctggatttcacttatactctctctcctggctctcagctcaggggccatttcccaggctgttgtgactcaggaatctgcactcaccacatcacctggtgaaacagtcacactcacttgtcgctcaagtactggggctgttacaactagtaatcatgccaactgggtccaagaaaaaccagatcctttattcactggtctattaggtgataccaacaaccgagctccaggtgttcctgccagattctcaggctccctgattggagacaaggctgccctcaccatcacaggggcacagcctgaggatgaggcaatatatttctgtgctctatggtacagtaaccactgggtgttcggtggaggaaccaaactgattgtcctg

SEQ ID NO: 53 - protein, 128 aa, Mus musculus
MAWISLILSLLALSSGAISQAVVTQESALTTSPGETVTLTCRSSTGAVTTSNHANWVQEKPDPLFTGLLGDTNNRAPGVPARFSGSLIGDKAALTITGAQPEDEAIYFCALWYSNHWVFGGGTKLIVL

SEQ ID NO: 54 - DNA, 327 bp, Mus musculus
caggctgttgtgactcaggaatctgcactcaccacatcacctggtgaaacagtcacactcacttgtcgctcaagtactggggctgttacaactagtaatcatgccaactgggtccaagaaaaaccagatcctttattcactggtctattaggtgataccaacaaccgagctccaggtgttcctgccagattctcaggctccctgattggagacaaggctgccctcaccatcacaggggcacagcctgaggatgaggcaatatatttctgtgctctatggtacagtaaccactgggtgttcggtggaggaaccaaactgattgtcctg

SEQ ID NO: 55 - protein, 109 aa, Mus musculus
QAVVTQESALTTSPGETVTLTCRSSTGAVTTSNHANWVQEKPDPLFTGLLGDTNNRAPGVPARFSGSLIGDKAALTITGAQPEDEAIYFCALWYSNHWVFGGGTKLIVL

SEQ ID NO: 56 - protein, 9 aa, Mus musculus
TGAVTTSNH

SEQ ID NO: 57 - protein, 9 aa, Mus musculus
ALWYSNHWV

SEQ ID NO: 58 - DNA, 408 bp, Mus musculus
atggaatgtaactggatacttccttttattctgtcagtaacttcaggtgtctactcacagtttcagctccagcagtctggggctgaggtggctagacctgggtcttcagtgaaattgtcctgcagggcttctggctacacctcaactcgctactgggtgcagtgggtaaaacagagacctgggcagggtctggaatggattggggctatttatcctggagatggtgatacttggtacactcagagattcaaggacaaggccacattgactgcagataaaacctccagcactgcctacatgcaactcagcagcttggcatctgaggactctgcggtctattactgtgcaagcgtctcccggtggttcttcgctgtctggggcgcagggaccacggtcaccgtctcctca

SEQ ID NO: 59 - protein, 136 aa, Mus musculus
MECNWILPFILSVTSGVYSQFQLQQSGAEVARPGSSVKLSCRASGYTSTRYWVQWVKQRPGQGLEWIGAIYPGDGDTWYTQRFKDKATLTADKTSSTAYMQLSSLASEDSAVYYCASVSRWFFAVWGAGTTVTVSS

SEQ ID NO: 60 - DNA, 351 bp, Mus musculus
cagtttcagctccagcagtctggggctgaggtggctagacctgggtcttcagtgaaattgtcctgcagggcttctggctacacctcaactcgctactgggtgcagtgggtaaaacagagacctgggcagggtctggaatggattggggctatttatcctggagatggtgatacttggtacactcagagattcaaggacaaggccacattgactgcagataaaacctccagcactgcctacatgcaactcagcagcttggcatctgaggactctgcggtctattactgtgcaagcgtctcccggtggttcttcgctgtctggggcgcagggaccacggtcaccgtctcctca

SEQ ID NO: 61 - protein, 117 aa, Mus musculus
QFQLQQSGAEVARPGSSVKLSCRASGYTSTRYWVQWVKQRPGQGLEWIGAIYPGDGDTWYTQRFKDKATLTADKTSSTAYMQLSSLASEDSAVYYCASVSRWFFAVWGAGTTVTVSS

SEQ ID NO: 62 - protein, 8 aa, Mus musculus
GYTSTRYW

SEQ ID NO: 63 - protein, 8 aa, Mus musculus
IYPGDGDT

SEQ ID NO: 64 - protein, 10 aa, Mus musculus
ASVSRWFFAV

SEQ ID NO: 65 - DNA, 384 bp, Mus musculus
atggcctggatttcacttatactctctctcctggctctcagctcaggggccatttcccaggctattgtgactcaggaatctgcactcaccacatcacctggtgaaacagtcacactcacttgtcgctcaagtactggggctgttacaactagtaaatatgccaactgggtccaagaaaaaccagatcatttattcactggtctaataggtggtaccaacaaccgagctccaggtgttcctgccagattctcaggctccctgattggagacaaggctgccctcaccatcacaggggcacagactgaggatgaggcaatatatttctgtgctctatggtacagcaaccactgggtgttcggtggaggaaccaaactgactgtccta

SEQ ID NO: 66 - protein, 128 aa, Mus musculus
MAWISLILSLLALSSGAISQAIVTQESALTTSPGETVTLTCRSSTGAVTTSKYANWVQEKPDHLFTGLIGGTNNRAPGVPARFSGSLIGDKAALTITGAQTEDEAIYFCALWYSNHWVFGGGTKLTVL

SEQ ID NO: 67 - DNA, 327 bp, Mus musculus
caggctattgtgactcaggaatctgcactcaccacatcacctggtgaaacagtcacactcacttgtcgctcaagtactggggctgttacaactagtaaatatgccaactgggtccaagaaaaaccagatcatttattcactggtctaataggtggtaccaacaaccgagctccaggtgttcctgccagattctcaggctccctgattggagacaaggctgccctcaccatcacaggggcacagactgaggatgaggcaatatatttctgtgctctatggtacagcaaccactgggtgttcggtggaggaaccaaactgactgtccta

SEQ ID NO: 68 - protein, 109 aa, Mus musculus
QAIVTQESALTTSPGETVTLTCRSSTGAVTTSKYANWVQEKPDHLFTGLIGGTNNRAPGVPARFSGSLIGDKAALTITGAQTEDEAIYFCALWYSNHWVFGGGTKLTVL

SEQ ID NO: 69 - protein, 9 aa, Mus musculus
TGAVTTSKY

SEQ ID NO: 70 - protein, 9 aa, Mus musculus
ALWYSNHWV

SEQ ID NO: 71 - DNA, 417 bp, Mus musculus
atggaatggagttggatatttctctttctcctgtcaggaactgcaggtgtccactctgaggtccagctgcagcagtctggacctgagctggtaaagcctggggcttcagtgaagatgtcctgcaaggcttctggatacacattcactaactatgctatgtactgggtgaagcagaaacctgggcagggccttgagtggattggatatattaatcctttcaatgacggtactaagaacaatgagaagttcaaagggaaggccacactgacttcagacaaatcctccagcacagcctacatggagctcagcagcctgacctctgaggactctgcggtctattactgtgcaagatattattactacggtagcaaggctatggactactggggtcaaggaaccgcagtcaccgtctcctca

SEQ ID NO: 72 - protein, 139 aa, Mus musculus; identical to SEQ ID NO: 7

SEQ ID NO: 73 - DNA, 360 bp, Mus musculus
gaggtccagctgcagcagtctggacctgagctggtaaagcctggggcttcagtgaagatgtcctgcaaggcttctggatacacattcactaactatgctatgtactgggtgaagcagaaacctgggcagggccttgagtggattggatatattaatcctttcaatgacggtactaagaacaatgagaagttcaaagggaaggccacactgacttcagacaaatcctccagcacagcctacatggagctcagcagcctgacctctgaggactctgcggtctattactgtgcaagatattattactacggtagcaaggctatggactactggggtcaaggaaccgcagtcaccgtctcctca

SEQ ID NO: 74 - protein, 120 aa, Mus musculus; identical to SEQ ID NO: 9

SEQ ID NO: 75 - protein, 8 aa, Mus musculus
GYTFTNYA

SEQ ID NO: 76 - protein, 8 aa, Mus musculus
INPFNDGT

SEQ ID NO: 77 - protein, 13 aa, Mus musculus
ARYYYYGSKAMDY

SEQ ID NO: 78 - DNA, 384 bp, Mus musculus
atggcctggatttcacttatactctctctcctggctctcagctcaggggccatttcccaggctgttgtgactcaggaatctgcactcaccacatcacctggtgaaacagtcacactcacttgtcgctcaaatactggggctgttagaattagtaactatgccaactgggtccgagaaaaaccagatcatttattcactggtctaataggtggtaccaacaaccgagctccaggtgttcctgccagattctcaggctccctgattggagacaaggctgccctcaccatcacaggggcacagactgatgatgaggcaatatatttctgtgctctatggaacagcaaccattgggtgttcggtggaggaaccaaactgactgtccta

SEQ ID NO: 79 - protein, 128 aa, Mus musculus
MAWISLILSLLALSSGAISQAVVTQESALTTSPGETVTLTCRSNTGAVRISNYANWVREKPDHLFTGLIGGTNNRAPGVPARFSGSLIGDKAALTITGAQTDDEAIYFCALWNSNHWVFGGGTKLTVL

SEQ ID NO: 80 - DNA, 327 bp, Mus musculus
caggctgttgtgactcaggaatctgcactcaccacatcacctggtgaaacagtcacactcacttgtcgctcaaatactggggctgttagaattagtaactatgccaactgggtccgagaaaaaccagatcatttattcactggtctaataggtggtaccaacaaccgagctccaggtgttcctgccagattctcaggctccctgattggagacaaggctgccctcaccatcacaggggcacagactgatgatgaggcaatatatttctgtgctctatggaacagcaaccattgggtgttcggtggaggaaccaaactgactgtccta

SEQ ID NO: 81 - protein, 109 aa, Mus musculus
QAVVTQESALTTSPGETVTLTCRSNTGAVRISNYANWVREKPDHLFTGLIGGTNNRAPGVPARFSGSLIGDKAALTITGAQTDDEAIYFCALWNSNHWVFGGGTKLTVL

SEQ ID NO: 82 - protein, 9 aa, Mus musculus
TGAVRISNY

SEQ ID NO: 83 - protein, 9 aa, Mus musculus
ALWNSNHWV

SEQ ID NO: 84 - protein, 189 aa, Mus musculus
MAALRMLWMGLVLLGLLGFPQTPAQGHDTVQPNFQQDKFLGRWYSAGLASNSSWFREKKAVLYMCKTVVAPSTEGGLNLTSTFLRKNQCETKIMVLQPAGAPGHYTYSSPHSGSIHSVSVVEANYDEYALLFSRGTKGPGQDFRMATLYSRTQTLKDELKEKFTTFSKAQGLTEEDIVFLPQPDKCIQE